European Patent Application EP 4 759 823 A1, published June 17, 2026. Title: Peptide Having Activity of Promoting Hair Growth and Inhibiting Hair Loss and Uses Thereof. Applicant: CAREGEN CO., LTD. The sequence listing filed with the application follows.

SEQUENCE LISTING (45 sequences)

SEQ ID NO: 1 - protein, 4 aa, synthetic construct
DRFF

SEQ ID NO: 2 - DNA, 20 bp, synthetic construct
  source 1..20: mol_type = other DNA
tgctggtgatgggagttgta

SEQ ID NO: 3 - DNA, 20 bp, synthetic construct
  source 1..20: mol_type = other DNA
cctccaagtagcagccaaag

SEQ ID NO: 4 - DNA, 20 bp, synthetic construct
  source 1..20: mol_type = other DNA
caatgcctctggttcccctt

SEQ ID NO: 5 - DNA, 20 bp, synthetic construct
  source 1..20: mol_type = other DNA
cccctcgaggatttcgacag

SEQ ID NO: 6 - DNA, 22 bp, synthetic construct
  source 1..22: mol_type = other DNA
tctgtcgaacacagtggtacct

SEQ ID NO: 7 - DNA, 23 bp, synthetic construct
  source 1..23: mol_type = other DNA
gtgtgtccatttagctgatgcat

SEQ ID NO: 8 - DNA, 22 bp, synthetic construct
  source 1..22: mol_type = other DNA
atgaactttctgggtcttgggt

SEQ ID NO: 9 - DNA, 22 bp, synthetic construct
  source 1..22: mol_type = other DNA
tggccttggtgaggtttgatcc

SEQ ID NO: 10 - DNA, 20 bp, synthetic construct
  source 1..20: mol_type = other DNA
ggagccaaaagggtcatcat

SEQ ID NO: 11 - DNA, 20 bp, synthetic construct
  source 1..20: mol_type = other DNA
gtgatggcatggactgtggt

SEQ ID NO: 12 - DNA, 20 bp, synthetic construct
  source 1..20: mol_type = other DNA
ccagctattgtaacacctca

SEQ ID NO: 13 - DNA, 20 bp, synthetic construct
  source 1..20: mol_type = other DNA
ttcagatgtaggcagctgtc

SEQ ID NO: 14 - DNA, 28 bp, synthetic construct
  source 1..28: mol_type = other DNA
accttcgttgccctctgtgccacagatg

SEQ ID NO: 15 - DNA, 21 bp, synthetic construct
  source 1..21: mol_type = other DNA
aggcccggaggcagtccgggt

SEQ ID NO: 16 - DNA, 25 bp, synthetic construct
  source 1..25: mol_type = other DNA
accagcagcgactctgaggaggaac

SEQ ID NO: 17 - DNA, 26 bp, synthetic construct
  source 1..26: mol_type = other DNA
tgaccctcttggcagcaggatagtcc

SEQ ID NO: 18 - DNA, 20 bp, synthetic construct
  source 1..20: mol_type = other DNA
gatcatcgagctgagacgca

SEQ ID NO: 19 - DNA, 20 bp, synthetic construct
  source 1..20: mol_type = other DNA
ctggccccagggtatctagt

SEQ ID NO: 20 - DNA, 20 bp, synthetic construct
  source 1..20: mol_type = other DNA
cgcggcgtatccgtgtcctc

SEQ ID NO: 21 - DNA, 24 bp, synthetic construct
  source 1..24: mol_type = other DNA
agcctgttccgtctcaaacttggt

SEQ ID NO: 22 - DNA, 20 bp, synthetic construct
  source 1..20: mol_type = other DNA
ccaaatccgcaccaaggtca

SEQ ID NO: 23 - DNA, 21 bp, synthetic construct
  source 1..21: mol_type = other DNA
gtattgattgccaggaggggg

SEQ ID NO: 24 - DNA, 20 bp, synthetic construct
  source 1..20: mol_type = other DNA
ccctcaaggatgccaggaac

SEQ ID NO: 25 - DNA, 19 bp, synthetic construct
  source 1..19: mol_type = other DNA
cactgctacctccggcaag

SEQ ID NO: 26 - DNA, 20 bp, synthetic construct
  source 1..20: mol_type = other DNA
cggtcaagtcggaaaattca

SEQ ID NO: 27 - DNA, 20 bp, synthetic construct
  source 1..20: mol_type = other DNA
gaggagctgggatgtggtaa

SEQ ID NO: 28 - DNA, 20 bp, synthetic construct
  source 1..20: mol_type = other DNA
gccgtctatacggacatgcc

SEQ ID NO: 29 - DNA, 20 bp, synthetic construct
  source 1..20: mol_type = other DNA
gcagtacacctgactgtccc

SEQ ID NO: 30 - DNA, 20 bp, synthetic construct
  source 1..20: mol_type = other DNA
caggactgggtgatggtgtc

SEQ ID NO: 31 - DNA, 20 bp, synthetic construct
  source 1..20: mol_type = other DNA
tctgagggtgagagcctgaa

SEQ ID NO: 32 - DNA, 20 bp, synthetic construct
  source 1..20: mol_type = other DNA
gagaccaaagaggcgttgga

SEQ ID NO: 33 - DNA, 20 bp, synthetic construct
  source 1..20: mol_type = other DNA
ggctagttttcacgctggtc

SEQ ID NO: 34 - DNA, 20 bp, synthetic construct
  source 1..20: mol_type = other DNA
ccagcaagacggagatcaca

SEQ ID NO: 35 - DNA, 20 bp, synthetic construct
  source 1..20: mol_type = other DNA
gaagaggcttccctgatggc

SEQ ID NO: 36 - DNA, 20 bp, synthetic construct
  source 1..20: mol_type = other DNA
aagctgcaacgaaaacgacg

SEQ ID NO: 37 - DNA, 20 bp, synthetic construct
  source 1..20: mol_type = other DNA
ggtggggctagtcaagtctg

SEQ ID NO: 38 - DNA, 20 bp, synthetic construct
  source 1..20: mol_type = other DNA
cctatccccgggactaagac

SEQ ID NO: 39 - DNA, 20 bp, synthetic construct
  source 1..20: mol_type = other DNA
atgctcttcaggggcaacac

SEQ ID NO: 40 - DNA, 20 bp, synthetic construct
  source 1..20: mol_type = other DNA
tggaccagctaaccaacgac

SEQ ID NO: 41 - DNA, 20 bp, synthetic construct
  source 1..20: mol_type = other DNA
gtcattgttccggttggcag

SEQ ID NO: 42 - DNA, 20 bp, synthetic construct
  source 1..20: mol_type = other DNA
ccgttctccccaggaaactt

SEQ ID NO: 43 - DNA, 20 bp, synthetic construct
  source 1..20: mol_type = other DNA
tgcagcgatcaggtcgttta

SEQ ID NO: 44 - DNA, 20 bp, synthetic construct
  source 1..20: mol_type = other DNA
cccagccaacctatgaggag

SEQ ID NO: 45 - DNA, 20 bp, synthetic construct
  source 1..20: mol_type = other DNA
cttgaggagaccagcaccac